European Patent Specification EP 3 546 581 B1, published April 1, 2026. Title: Microorganism of genus corynebacterium producing L-arginine and method for producing L-arginine using the same. Applicant: CJ CheilJedang Corporation. The sequence listing filed with the application follows.

SEQUENCE LISTING (11 sequences)

SEQ ID NO: 1 - protein, 356 aa, Corynebacterium glutamicum
VLLRAEEVVRQGQRGIKLHVEAQHEHHHHRHLSTIKELLVNADIPAQTKQDALGVFELIAIAEGKVHGIEPEKIHFHEVGAWDSIADIVGVCEAIRQLNPGLIAASPIALGFGRIKAAHGDIPVPVPAVAELVKGWPTQTGALMESTEPVGELATPTGVALIRHFATQDGPFPGGIINEVGIGAGTKDTAGRPNVVRAVLFSTSGKAASNPDTRTLVQLEANVDDQDPRLWPGVIESLFAAGAVAAWLTPILMKKGRPAHTVSALVDSSEVEAVKTALFAATTTFGVRSWEVQREGLDRRFEQVEVDGRTINIKIGSRNGHDISAQPEFEDIRSAAVALGISEREVVARIPQGTTE

SEQ ID NO: 2 - DNA, 1071 bp, Corynebacterium glutamicum
gtgcttttgagagcagaagaggtagtgcgccaaggccaacgaggcatcaaactacatgtagaagcacaacatgaacaccaccatcaccgccatttgagcaccattaaagaactgcttgtcaatgctgacatccctgcacaaaccaagcaggatgccttaggcgtttttgaactcatcgctatcgctgaaggaaaagtccacggcatcgagccggagaaaatccacttccatgaggtaggagcttgggattccatcgcagacattgtgggtgtgtgcgaagcgatcaggcagcttaacccaggtttgattgctgcatctccgattgctttaggattcggacgcatcaaggcagctcacggagacattccagtgccagttccagcagtggcagagctggtgaaaggctggcccacccaaaccggagctcttatggagagcaccgaacctgttggtgaattagccaccccaactggtgttgcgttgatccgtcactttgccacccaagatggccctttcccaggtggcatcatcaatgaagtcggtatcggcgcaggaactaaggacaccgcagggcgtcccaatgtggtgcgcgcggtcctgttcagcacctccggtaaggctgcctcaaacccagacacccgtaccctcgtgcaattggaagccaacgttgatgatcaagacccacggctgtggccaggagtaatagagagcctctttgccgctggcgcagtagctgcatggctgactccaattttgatgaagaagggccgtcctgcacatacggtgtcagcattggtggatagctccgaggtggaagcagtgaaaaccgcattatttgcagccaccacgacttttggggtcagatcatgggaagtccagcgagaagggttggatcgtcgtttcgaacaagtcgaggtggacggacgcaccatcaacatcaagattggctcccgaaatggccacgacatcagtgcacagcccgagtttgaagatattcggtctgcagcggtggccttgggaatttcagagagggaagttgtggcaagaattccgcaaggcaccactgagtaa

SEQ ID NO: 3 - DNA, 25 bp, Artificial Sequence
  Primer 1
acctacaacaaagctctcatcaacc

SEQ ID NO: 4 - DNA, 24 bp, Artificial Sequence
  Primer 2
ctaccctgtggaacacctacatct

SEQ ID NO: 5 - DNA, 29 bp, Artificial Sequence
  Primer 3
ccgctcgagacatcgaaatcgtaagggta

SEQ ID NO: 6 - DNA, 20 bp, Artificial Sequence
  Primer 4
cagcattgacaagcagttct

SEQ ID NO: 7 - DNA, 40 bp, Artificial Sequence
  Primer 5
agaactgcttgtcaatgctgggccctttcccaggtggcat

SEQ ID NO: 8 - DNA, 29 bp, Artificial Sequence
  Primer 6
ccgctcgagaaggccaccgctgcagaccg

SEQ ID NO: 9 - DNA, 30 bp, Artificial Sequence
  Primer 7
gatccacagtcccaatattctcgcttcttc

SEQ ID NO: 10 - DNA, 30 bp, Artificial Sequence
  Primer 8
gaagaagcgagaatattgggactgtggatc

SEQ ID NO: 11 - DNA, 29 bp, Artificial Sequence
  Primer 9
ccgctcgagcagcattgacaagcagttct